European Patent Specification EP 3 953 463 B1, published August 6, 2025. Title: Stabilized Variants. Applicant: Novozymes A/S. The sequence listing filed with the application follows.

SEQUENCE LISTING (201 sequences)

SEQ ID NO: 1 - protein, 278 aa, Thielavia terrestris [sequence omitted]

SEQ ID NO: 2 - protein, 283 aa, Humicola insolens
ADGRSTRYWDCCKPSCGWAKKAPVNQPVFSCNANFQRITDFDAKSGCEPGGVAYSCADQTPWAVNDDFALGFAATSIAGSNEAGWCCACYELTFTSGPVAGKKMVVQSTSTGGDLGSNHFDLNIPGGGVGIFDGCTPQFGGLPGQRYGGISSRNECDRFPDALKPGCYWRFDWFKNADNPSFSFRQVQCPAELVARTGCRRNDDGNFPAVQISSSTSSPVNQPTSTSTTSTSTTSSPPVQPTTPSGCTAERWAQCGGNGWSGCTTCVAGSTCTKINDWYHQCL

SEQ ID NO: 3 - protein, 295 aa, Staphylotrichum coccosporum
ADGKSTRYWDCCKPSCSWPGKASVNQPVFACSANFQRISDPNVKSGCDGGSAYACADQTPWAVNDNFSYGFAATSISGGNEASWCCGCYELTFTSGPVAGKTMVVQSTSTGGDLGTNHFDLAMPGGGVGIFDGCSPQFGGLAGDRYGGVSSRSQCDSFPAALKPGCYWRFDWFKNADNPTFTFRQVQCPSELVARTGCRRNDDGNFPVFTPPSGGQSSSSSSSSSAKPTSTSTSTTSTKATSTTSTASSQTSSSTGGGCAAQRWAQCGGIGFSGCTTCVSGTTCNKQNDWYSQCL

SEQ ID NO: 4 - protein, 277 aa, Acremonium thermophilum
ALDGKSTRYWDCCKPSCGWPGKASVNQPVFSCSADWQRISDFNAKSGCDGGSAYSCADQTPWAVNDNFSYGFAATAIAGGSESSWCCACYALTFNSGPVAGKTMVVQSTSTGGDLGSNQFDLAIPGGGVGIFNGCASQFGGLPGAQYGGISDRSQCSSFPAPLQPGCQWRFDWFQNADNPTFTFQRVQCPSELTSRTGCKRDDDASYPVFNPPSGGSPSTTSTTTSSPSGPTGNPPGGGGCTAQKWAQCGGTGFTGCTTCVSGTTCQVQNQWYSQCL

SEQ ID NO: 5 - protein, 212 aa, Artificial Sequence
  Catalytic domain of SEQ ID NO: 1
ASGSGQSTRYWDCCKPSCAWPGKAAVSQPVYACDANFQRLSDFNVQSGCNGGSAYSCADQTPWAVNDNLAYGFAATSIAGGSESSWCCACYALTFTSGPVAGKTMVVQSTSTGGDLGSNHFDIAMPGGGVGIFNGCSSQFGGLPGAQYGGISSRDQCDSFPAPLKPGCQWRFDWFQNADNPTFTFQQVQCPAEIVARSGCKRNDDSSFPVFT

SEQ ID NO: 6 - protein, 37 aa, Artificial Sequence
  carbohydrate binding module of SEQ ID NO: 1
CTSQKWAQCGGIGFSGCTTCVSGTTCQKLNDYYSQCL

SEQ ID NO: 7 - protein, 37 aa, Artificial Sequence
  carbohydrate binding module of SEQ ID NO: 2
CTAERWAQCGGNGWSGCTTCVAGSTCTKINDWYHQCL

SEQ ID NO: 8 - protein, 37 aa, Artificial sequence
  Carbohydrate binding module of SEQ ID NO: 3
CAAQRWAQCGGIGFSGCTTCVSGTTCNKQNDWYSQCL

SEQ ID NO: 9 - protein, 37 aa, Artificial Sequence
  Carbohydrate binding module of SEQ ID NO: 4
CTAQKWAQCGGTGFTGCTTCVSGTTCQVQNQWYSQCL

SEQ ID NO: 10 - protein, 311 aa, Artificial Sequence
  Synthetic Construct
AVPSTQTPWGIKSIYNDQSITKTTGGKGIKVAVLDTGVYTSHLDLAGSAEQCKDFTQSNPLVDGSCTDRQGHGTHVAGTVLAHGGSNGQGVYGVAPQAKLWAYKVLGDKGEGYSDDIAAAIRHVADEASRTGSKVVINMSLGSSAKDSLIASAVDYAYGKGVLIVAAAGNEGPKPNTIGYPAGFVNAVAVAALENVQEKGTYRVADFSSRGNPATAGDYIIQERDIEVSAPGASVESTWYTGGYNTISGTSMATPHVAGLAAKIWSANTSLSHSQLRTELQNRAKVYDIKGGIGAGPGDDYASGFGYPRVK

SEQ ID NO: 11 - protein, 269 aa, Bacillus lentus
AQSVPWGISRVQAPAAHNRGLTGSGVKVAVLDTGISTHPDLNIRGGASFVPGEPSTQDGNGHGTHVAGTIAALNNSIGVLGVAPSAELYAVKVLGASGSGSVSSIAQGLEWAGNNGMHVANLSLGSPSPSATLEQAVNSATSRGVLVVAASGNSGAGSISYPARYANAMAVGATDQNNNRASFSQYGAGLDIVAPGVNVQSTYPGSTYASLNGTSMATPHVAGAAALVKQKNPSWSNVQIRNHLKNTATSLGSTNLYGSGLVNAEAATR

SEQ ID NO: 12 - protein, 13 aa, Artificial Sequence
  Linker
TTPPTPTPTPTPG

SEQ ID NO: 13 - protein, 15 aa, Artificial Sequence
  Linker
TTPTPPTPTPTPTPG

SEQ ID NO: 14 - protein, 17 aa, Artificial Sequence
  Linker
TTPTPTPPTPTPTPTPG

SEQ ID NO: 15 - protein, 19 aa, Artificial Sequence
  Linker
TTPTPTPTPPTPTPTPTPG

SEQ ID NO: 16 - protein, 34 aa, Artificial Sequence
  Synthetic Construct
TPPTPPTPPTPPTPPTPPTPPTPPTPPTPPTPPG

SEQ ID NO: 17 - protein, 13 aa, Artificial Sequence
  Linker
TPTTPTTPTTPTG

SEQ ID NO: 18 - protein, 19 aa, Artificial Sequence
  Linker
TPTTPTTPTTPTTPTTPTG

SEQ ID NO: 19 - protein, 13 aa, Artificial Sequence
  Linker
SPSSPSSPSSPSG

SEQ ID NO: 20 - protein, 16 aa, Artificial Sequence
  Linker
SPSSPSSPSSPSSPSG

SEQ ID NO: 21 - protein, 16 aa, Artificial Sequence
  Linker
SPPSPPSPPSPPSPPG

SEQ ID NO: 22 - protein, 31 aa, Artificial Sequence
  Linker
SPPSPPSPPSPPSPPSPPSPPSPPSPPSPPG

SEQ ID NO: 23 - protein, 22 aa, Artificial Sequence
  Linker
PPSSPSSPSSPSSPSSPSSPSG

SEQ ID NO: 24 - protein, 5 aa, Artificial Sequence
  Linker
SPSPG

SEQ ID NO: 25 - protein, 11 aa, Artificial Sequence
  Linker
SPSPSPSPSPG

SEQ ID NO: 26 - protein, 11 aa, Artificial Sequence
  Linker
TPTPTPTPTPG

SEQ ID NO: 27 - protein, 4 aa, Artificial Sequence
  Linker
PPPP

SEQ ID NO: 28 - protein, 5 aa, Artificial Sequence
  Linker
PPPPP

SEQ ID NO: 29 - protein, 6 aa, Artificial Sequence
  Linker
PPPPPP

SEQ ID NO: 30 - protein, 8 aa, Artificial Sequence
  Linker
PPPPPPPG

SEQ ID NO: 31 - protein, 7 aa, Artificial Sequence
  Linker
PPPPPPP

SEQ ID NO: 32 - protein, 9 aa, Artificial Sequence
  Linker
PPPPPPPPG

SEQ ID NO: 33 - protein, 10 aa, Artificial Sequence
  Linker
PPPPPPPPPG

SEQ ID NO: 34 - protein, 11 aa, Artificial Sequence
  Linker
PPPPPPPPPPG

SEQ ID NO: 35 - protein, 12 aa, Artificial Sequence
  Linker
PPPPPPPPPPPG

SEQ ID NO: 36 - protein, 14 aa, Artificial Sequence
  Linker
PPPPPPPPPPPPPG

SEQ ID NO: 37 - protein, 9 aa, Artificial Sequence
  Linker
PEPTPEPTG

SEQ ID NO: 38 - protein, 13 aa, Artificial Sequence
  Linker
PEPTPEPTPEPTG

SEQ ID NO: 39 - protein, 17 aa, Artificial Sequence
  Linker
PEPTPEPTPEPTPEPTG

SEQ ID NO: 40 - protein, 21 aa, Artificial Sequence
  Linker
PEPTPEPTPEPTPEPTPEPTG

SEQ ID NO: 41 - protein, 17 aa, Artificial Sequence
  Linker
PSPTPSPTPSPTPSPTG

SEQ ID NO: 42 - protein, 21 aa, Artificial Sequence
  Linker
PSPTPSPTPSPTPSPTPSPTG

SEQ ID NO: 43 - protein, 9 aa, Artificial Sequence
  Linker
PQPTPQPTG

SEQ ID NO: 44 - protein, 9 aa, Artificial Sequence
  Linker
PDPTPDPTG

SEQ ID NO: 45 - protein, 9 aa, Artificial Sequence
  Linker
PRPTPEPTG

SEQ ID NO: 46 - protein, 9 aa, Artificial Sequence
  Linker
PQPTPEPTG

SEQ ID NO: 47 - protein, 11 aa, Artificial Sequence
  Linker
PSPNSPNSPNG

SEQ ID NO: 48 - protein, 9 aa, Artificial Sequence
  Linker
PEPTPRPTG

SEQ ID NO: 49 - protein, 29 aa, Artificial Sequence
  Linker
PQPTPEPTPQPTPEPTPQPTPEPTPQPTG

SEQ ID NO: 50 - protein, 13 aa, Artificial Sequence
  Linker
PDPTPDPTPDPTG

SEQ ID NO: 51 - protein, 17 aa, Artificial Sequence
  Linker
PQPTPQPTPQPTPQPTG

SEQ ID NO: 52 - protein, 17 aa, Artificial Sequence
  Linker
PQPTPEPTPQPTPEPTG

SEQ ID NO: 53 - protein, 11 aa, Artificial Sequence
  Linker
SPSPSPSPPPG

SEQ ID NO: 54 - protein, 11 aa, Artificial Sequence
  Linker
SPSPSPSPDPG

SEQ ID NO: 55 - protein, 11 aa, Artificial Sequence
  Linker
SPSPSPSPKPG

SEQ ID NO: 56 - protein, 11 aa, Artificial Sequence
  Linker
SPSPSPSPAPG

SEQ ID NO: 57 - protein, 12 aa, Artificial Sequence
  Linker
SPSPSPSPSPSG

SEQ ID NO: 58 - protein, 10 aa, Artificial Sequence
  Linker
SPSPSPSPSP

SEQ ID NO: 59 - protein, 11 aa, Artificial Sequence
  Linker
SPSPSPSPSPS

SEQ ID NO: 60 - protein, 11 aa, Artificial Sequence
  Linker
SPSPSPSPSPP

SEQ ID NO: 61 - protein, 11 aa, Artificial Sequence
  Linker
SPSPSPSPSPE

SEQ ID NO: 62 - protein, 11 aa, Artificial Sequence
  Linker
SPSPSPSPSPN

SEQ ID NO: 63 - protein, 12 aa, Artificial Sequence
  Linker
SPSPSPSPSPGG

SEQ ID NO: 64 - protein, 11 aa, Artificial Sequence
  Linker
SPSPSPSPSPK

SEQ ID NO: 65 - protein, 9 aa, Artificial Sequence
  Linker
PEPTPEPTP

SEQ ID NO: 66 - protein, 9 aa, Artificial Sequence
  Linker
PEPTPEPTR

SEQ ID NO: 67 - protein, 13 aa, Artificial Sequence
  Linker
PEPTPEPTPEPTP

SEQ ID NO: 68 - protein, 21 aa, Artificial Sequence
  Linker
PEPTPEPTPEPTPEPTPSPTG

SEQ ID NO: 69 - protein, 21 aa, Artificial Sequence
  Linker
PEPTPEPTPEPTPEPTPTPTG

SEQ ID NO: 70 - protein, 21 aa, Artificial Sequence
  Linker
PEPTPEPTPEPTPEPTPGPTG

SEQ ID NO: 71 - protein, 21 aa, Artificial Sequence
  Linker
PEPTPEPTPEPTPEPTPDPTG

SEQ ID NO: 72 - protein, 20 aa, Artificial Sequence
  Linker
PEPTPEPTPEPTPEPTPETG

SEQ ID NO: 73 - protein, 21 aa, Artificial Sequence
  Linker
PEPTPEPTPEPTPEPTPEPTD

SEQ ID NO: 74 - protein, 9 aa, Artificial Sequence
  Linker
PEPTPEPTE

SEQ ID NO: 75 - protein, 19 aa, Artificial Sequence
  Linker
PEPTPEPTPEPTPEPTPEP

SEQ ID NO: 76 - protein, 20 aa, Artificial Sequence
  Linker
PEPTPEPTPEPTPEPTPSPT

SEQ ID NO: 77 - protein, 21 aa, Artificial Sequence
  Linker
PEPTPEPTPEPTPEPTPRPTT

SEQ ID NO: 78 - protein, 21 aa, Artificial Sequence
  Linker
PEPTPEPTPEPTPEPTPEPTT

SEQ ID NO: 79 - protein, 20 aa, Artificial Sequence
  Linker
PEPTPEPTPEPTPEPTPEPT

SEQ ID NO: 80 - protein, 21 aa, Artificial Sequence
  Linker
PEPTPEPTPEPTPEPTPEPTS

SEQ ID NO: 81 - protein, 21 aa, Artificial Sequence
  Linker
PEPTPEPTPEPTPEPTPEPTR

SEQ ID NO: 82 - protein, 29 aa, Artificial Sequence
  Linker
PPPGGPGGPGTPTSTAPGSGPTSPGGGSG

SEQ ID NO: 83 - protein, 29 aa, Artificial Sequence
  Linker
PPPGGPGGTGTPTSTAPGSGPTSPGGGSG

SEQ ID NO: 84 - protein, 29 aa, Artificial Sequence
  Linker
PPSGGPGGPGTPTSTAPGSGPTSPGGGSG

SEQ ID NO: 85 - protein, 17 aa, Artificial Sequence
  Linker
PEPTPRPTPEPTPRPTG

SEQ ID NO: 86 - protein, 17 aa, Artificial Sequence
  Linker
PKPTPEPTPKPTPEPTG

SEQ ID NO: 87 - protein, 17 aa, Artificial Sequence
  Linker
PEPTPKPTPEPTPKPTG

SEQ ID NO: 88 - protein, 17 aa, Artificial Sequence
  Linker
PEPTPQPTPEPTPQPTG

SEQ ID NO: 89 - protein, 13 aa, Artificial Sequence
  Linker
PRPTPEPTPRPTG

SEQ ID NO: 90 - protein, 13 aa, Artificial Sequence
  Linker
PKPTPEPTPKPTG

SEQ ID NO: 91 - protein, 9 aa, Artificial Sequence
  Linker
PEPTPQPTG

SEQ ID NO: 92 - protein, 9 aa, Artificial Sequence
  Linker
PEPTPQPTG

SEQ ID NO: 93 - protein, 7 aa, Artificial Sequence
  Linker
TPPTPPG

SEQ ID NO: 94 - protein, 7 aa, Artificial Sequence
  Linker
SPSSPSG

SEQ ID NO: 95 - protein, 10 aa, Artificial Sequence
  Linker
SPSSPSSPSG

SEQ ID NO: 96 - protein, 7 aa, Artificial Sequence
  Linker
TPTTPTG

SEQ ID NO: 97 - protein, 10 aa, Artificial Sequence
  Linker
TPTTPTTPTG

SEQ ID NO: 98 - protein, 4 aa, Artificial Sequence
  Linker
  misc_feature (2)..(2): Xaa = any amino acid
  misc_feature (4)..(4): Xaa = any amino acid
PXPX

SEQ ID NO: 99 - protein, 4 aa, Artificial Sequence
  Linker
  misc_feature (1)..(1): Xaa = any amino acid
  misc_feature (3)..(3): Xaa = any amino acid
XPXP

SEQ ID NO: 100 - protein, 6 aa, Artificial Sequence
  Linker
  misc_feature (1)..(1): Xaa = any amino acid
  misc_feature (3)..(3): Xaa = any amino acid
  misc_feature (4)..(4): Xaa = any amino acid
  misc_feature (6)..(6): Xaa = any amino acid
XPXXPX

SEQ ID NO: 101 - protein, 6 aa, Artificial Sequence
  Linker
  misc_feature (1)..(1): Xaa = any amino acid
  misc_feature (2)..(2): Xaa = any amino acid
  misc_feature (4)..(4): Xaa = any amino acid
  misc_feature (5)..(5): Xaa = any amino acid
XXPXXP

SEQ ID NO: 102 - protein, 4 aa, Artificial Sequence
  Linker
  misc_feature (2)..(2): Xaa = Ser, Thr, Arg, Lys, Asp, Glu, Asn, Gln
  misc_feature (4)..(4): Xaa = Ser, Thr, Arg, Lys, Asp, Glu
PXPX

SEQ ID NO: 103 - protein, 4 aa, Artificial Sequence
  Linker
PSPS

SEQ ID NO: 104 - protein, 4 aa, Artificial Sequence
  Linker
PSPT

SEQ ID NO: 105 - protein, 4 aa, Artificial Sequence
  Linker
PSPR

SEQ ID NO: 106 - protein, 4 aa, Artificial Sequence
  Linker
PSPK

SEQ ID NO: 107 - protein, 4 aa, Artificial Sequence
  Linker
PSPD

SEQ ID NO: 108 - protein, 4 aa, Artificial Sequence
  Linker
PSPE

SEQ ID NO: 109 - protein, 4 aa, Artificial Sequence
  Linker
  misc_feature (2)..(2): Xaa = Ser, Glu
PXPT

SEQ ID NO: 110 - protein, 6 aa, Artificial Sequence
  Linker
PPSPTP

SEQ ID NO: 111 - protein, 6 aa, Artificial Sequence
  Linker
PPTPTP

SEQ ID NO: 112 - protein, 6 aa, Artificial Sequence
  Linker
PPSPSP

SEQ ID NO: 113 - protein, 6 aa, Artificial Sequence
  Linker
SPPPTP

SEQ ID NO: 114 - protein, 6 aa, Artificial Sequence
  Linker
SPTPPP

SEQ ID NO: 115 - protein, 6 aa, Artificial Sequence
  Linker
SPPPPP

SEQ ID NO: 116 - protein, 6 aa, Artificial Sequence
  Linker
SPTPTP

SEQ ID NO: 117 - protein, 6 aa, Artificial Sequence
  Linker
TPPPSP

SEQ ID NO: 118 - protein, 6 aa, Artificial Sequence
  Linker
TPSPPP

SEQ ID NO: 119 - protein, 6 aa, Artificial Sequence
  Linker
TPPPPP

SEQ ID NO: 120 - protein, 6 aa, Artificial Sequence
  Linker
TPSPSP

SEQ ID NO: 121 - protein, 8 aa, Artificial Sequence
  Linker
PSPTPEPT

SEQ ID NO: 122 - protein, 16 aa, Artificial Sequence
  Linker
PSPTPEPTPSPTPEPT

SEQ ID NO: 123 - protein, 8 aa, Artificial Sequence
  Linker
PEPTPSPT

SEQ ID NO: 124 - protein, 12 aa, Artificial Sequence
  Linker
PEPTPSPTPSPT

SEQ ID NO: 125 - protein, 4 aa, Artificial Sequence
  Linker
PEPT

SEQ ID NO: 126 - protein, 6 aa, Artificial Sequence
  Linker
SPPEPT

SEQ ID NO: 127 - protein, 6 aa, Artificial Sequence
  Linker
SPPSPT

SEQ ID NO: 128 - protein, 6 aa, Artificial Sequence
  Linker
PSPEPT

SEQ ID NO: 129 - protein, 6 aa, Artificial Sequence
  Linker
PSPSPT

SEQ ID NO: 130 - protein, 4 aa, Artificial Sequence
  Linker
SPSP

SEQ ID NO: 131 - protein, 6 aa, Artificial Sequence
  Linker
SPSPSP

SEQ ID NO: 132 - protein, 8 aa, Artificial Sequence
  Linker
SPSPSPSP

SEQ ID NO: 133 - protein, 12 aa, Artificial Sequence
  Linker
SPSPSPSPSPSP

SEQ ID NO: 134 - protein, 14 aa, Artificial Sequence
  Linker
SPSPSPSPSPSPSP

SEQ ID NO: 135 - protein, 16 aa, Artificial Sequence
  Linker
SPSPSPSPSPSPSPSP

SEQ ID NO: 136 - protein, 8 aa, Artificial Sequence
  Linker
PPPPPPPP

SEQ ID NO: 137 - protein, 9 aa, Artificial Sequence
  Linker
PPPPPPPPP

SEQ ID NO: 138 - protein, 10 aa, Artificial Sequence
  Linker
PPPPPPPPPP

SEQ ID NO: 139 - protein, 11 aa, Artificial Sequence
  Linker
PPPPPPPPPPP

SEQ ID NO: 140 - protein, 12 aa, Artificial Sequence
  Linker
PPPPPPPPPPPP

SEQ ID NO: 141 - protein, 13 aa, Artificial Sequence
  Linker
PPPPPPPPPPPPP

SEQ ID NO: 142 - protein, 14 aa, Artificial Sequence
  Linker
PPPPPPPPPPPPPP

SEQ ID NO: 143 - protein, 15 aa, Artificial Sequence
  Linker
PPPPPPPPPPPPPPP

SEQ ID NO: 144 - protein, 8 aa, Artificial Sequence
  Linker
PEPTPEPT

SEQ ID NO: 145 - protein, 12 aa, Artificial Sequence
  Linker
PEPTPEPTPEPT

SEQ ID NO: 146 - protein, 16 aa, Artificial Sequence
  Linker
PEPTPEPTPEPTPEPT

SEQ ID NO: 147 - protein, 8 aa, Artificial Sequence
  Linker
PSPTPSPT

SEQ ID NO: 148 - protein, 12 aa, Artificial Sequence
  Linker
PSPTPSPTPSPT

SEQ ID NO: 149 - protein, 16 aa, Artificial Sequence
  Linker
PSPTPSPTPSPTPSPT

SEQ ID NO: 150 - protein, 20 aa, Artificial Sequence
  Linker
PSPTPSPTPSPTPSPTPSPT

SEQ ID NO: 151 - protein, 6 aa, Artificial Sequence
  Linker
SPSSPS

SEQ ID NO: 152 - protein, 9 aa, Artificial Sequence
  Linker
SPSSPSSPS

SEQ ID NO: 153 - protein, 12 aa, Artificial Sequence
  Linker
SPSSPSSPSSPS

SEQ ID NO: 154 - protein, 15 aa, Artificial Sequence
  Linker
SPSSPSSPSSPSSPS

SEQ ID NO: 155 - protein, 6 aa, Artificial Sequence
  Linker
TPTTPT

SEQ ID NO: 156 - protein, 9 aa, Artificial Sequence
  Linker
TPTTPTTPT

SEQ ID NO: 157 - protein, 12 aa, Artificial Sequence
  Linker
TPTTPTTPTTPT

SEQ ID NO: 158 - protein, 15 aa, Artificial Sequence
  Linker
TPTTPTTPTTPTTPT

SEQ ID NO: 159 - protein, 16 aa, Artificial Sequence
  Linker
PEPTPRPTPEPTPRPT

SEQ ID NO: 160 - protein, 16 aa, Artificial Sequence
  Linker
PEPTPKPTPEPTPKPT

SEQ ID NO: 161 - protein, 16 aa, Artificial Sequence
  Linker
PEPTPQPTPEPTPQPT

SEQ ID NO: 162 - protein, 12 aa, Artificial Sequence
  Linker
PRPTPEPTPRPT

SEQ ID NO: 163 - protein, 12 aa, Artificial Sequence
  Linker
PKPTPEPTPKPT

SEQ ID NO: 164 - protein, 8 aa, Artificial Sequence
  Linker
PEPTPQPT

SEQ ID NO: 165 - protein, 12 aa, Artificial Sequence
  Linker
PEPTPQPTPEPT

SEQ ID NO: 166 - protein, 12 aa, Artificial Sequence
  Linker
TTPPTPTPTPTP

SEQ ID NO: 167 - protein, 14 aa, Artificial Sequence
  Linker
TTPTPPTPTPTPTP

SEQ ID NO: 168 - protein, 16 aa, Artificial Sequence
  Linker
TTPTPTPPTPTPTPTP

SEQ ID NO: 169 - protein, 33 aa, Artificial Sequence
  Linker
TPPTPPTPPTPPTPPTPPTPPTPPTPPTPPTPP

SEQ ID NO: 170 - protein, 13 aa, Artificial Sequence
  Linker
PPPPPPPPPPPPG

SEQ ID NO: 171 - protein, 15 aa, Artificial Sequence
  Linker
PPPPPPPPPPPPPPG

SEQ ID NO: 172 - protein, 16 aa, Artificial Sequence
  Linker
PPPPPPPPPPPPPPPG

SEQ ID NO: 173 - protein, 37 aa, Chaetomium thermophilum
CTTQKWGQCGGIGYTGCTNCVAGTTCTQLNPWYSQCL

SEQ ID NO: 174 - protein, 37 aa, Chaetomium thermophilum
CTTQKWGQCGGIGYTGCTNCVAGTTCTELNPWYSQCL

SEQ ID NO: 175 - protein, 36 aa, Mycothermus thermophilus
CASKWGQCGGQGWAGPTCCEAGSTCTRQNEWYSQCL

SEQ ID NO: 176 - protein, 37 aa, Ovatospora medusarum
CTAARWQQCGGIGYSGCKACASPWTCQKLNDWYHQCL

SEQ ID NO: 177 - protein, 37 aa, Thermothelomyces heterothallica
CTVAKWGQCGGQGYSGCTVCAAGSTCQKTNDYYSQCL

SEQ ID NO: 178 - protein, 38 aa, Ovatospora medusarum
CSVQAFGQCGGTGYSGCTQCADGYTCKDVSPPYYSQCV

SEQ ID NO: 179 - protein, 37 aa, Thielavia arenaria
CTVAKWGQCGGLGWTGCTTCAAGSTCNKANDFYSQCV

SEQ ID NO: 180 - protein, 37 aa, Ovatospora medusarum
CTVAKYGQCGGNNYSGCTTCAAGSTCSRTNEYYSQCV

SEQ ID NO: 181 - protein, 37 aa, Chaetomium thermophile
CVTQKWAQCGGNGFSGCRTCASGSTCQVLNEWYSQCL

SEQ ID NO: 182 - protein, 37 aa, Chaetomium thermophile
CTVAKWAQCGGIGYSGCTTCEAGSTCRRTNDYYSQCV

SEQ ID NO: 183 - protein, 36 aa, Ovatospora medusarum
CTAAQWQQCGGTNFNGCTTCAAGYNCKLINEYYSQC

SEQ ID NO: 184 - protein, 38 aa, Chaetomium thermophile
CTAQRYQQCGGNGYTGCTNCAAGSTCSAVSPPYYSQCL

SEQ ID NO: 185 - protein, 37 aa, Thermothelomyces heterothallica
CTAAQWAQCGGINFTGCTTCASPYKCNFINDYYSQCY

SEQ ID NO: 186 - protein, 37 aa, Thielavia species
CVAQKWAQCGGSGFTGCTTCASGSTCQKQNDFYSQCL

SEQ ID NO: 187 - protein, 38 aa, Thielavia arenaria
CTVQRYGQCGGQGYTGCTTCASGSTCTGVSAPYYYQCI

SEQ ID NO: 188 - protein, 37 aa, Thielavia arenaria
CAAAKYGQCDGKNWNGCKSCVAGTTCRYQNDYYSQCL

SEQ ID NO: 189 - protein, 37 aa, Ovatospora medusarum
CVAQKWAQCGGKGFTGCKNCVSGTTCQEQNQWYSQCL

SEQ ID NO: 190 - protein, 37 aa, Thielavia arenaria
CNVAQWQQCGGSTYTGCTQCASPYTCKNINTYYSQCQ

SEQ ID NO: 191 - protein, 37 aa, Chaetomium thermophile
CTAARWGQCGGIGYSGCTACASPWTCQRISDWYHQCL

SEQ ID NO: 192 - protein, 36 aa, Adineta vaga
CNNIYNQCGGNGWNGTTNCCSGLSCVYKNSSYSQCL

SEQ ID NO: 193 - protein, 37 aa, Chaetomium species
CVAQKWAQCGGKGFTGCTTCVSGTTCKEHHEWYSQCL

SEQ ID NO: 194 - protein, 37 aa, Achaetomium strumarium
CTAQRWSQCGGNGFTGCTTCVSGTTCQKQNDWYSQCL

SEQ ID NO: 195 - protein, 36 aa, Chaetomium thermophile
CTVPQWAQCGGVNYTGCTTCAPGYTCKYTNDYYSQC

SEQ ID NO: 196 - protein, 37 aa, Ovatospora medusarum
CVSQKWAQCGGNGYTGCTQCVSGTTCNKLNDWYSQCL

SEQ ID NO: 197 - protein, 37 aa, Chaetomium olivicolor
CTAQKWAQCGGSGFSGCTSCVSGTTCQKQNDWYSQCL

SEQ ID NO: 198 - protein, 37 aa, Taifanglania major
CVAQKWAQCGGNGFTGCTTCVSGTTCTKSNDWYSQCL

SEQ ID NO: 199 - protein, 37 aa, Trichocladium asperum
CFAQKWAQCGGNGFTGCTSCVSGTTCQKQNDWYSQCL

SEQ ID NO: 200 - protein, 37 aa, Ovatospora brasiliensis
CVAQKWAQCGGNGFSGCTTCVSGSTCQKQNDWYSQCL

SEQ ID NO: 201 - protein, 262 aa, Artificial Sequence
  Synthetic Construct
ASGSGQSTRYWDCCKPSCAWPGKAAVSQPVYACDANFQRLSDFNVQSGCNGGSAYSCADQTPWAVNDNLAYGFAATSIAGGSESSWCCACYALTFTSGPVAGKTMVVQSTSTGGDLGSNHFDIAMPGGGVGIFNGCSSQFGGLPGAQYGGISSRDQCDSFPAPLKPGCQWRFDWFQNADNPTFTFQQVQCPAEIVARSGCKRNDDSSFPVFTTTPPTPTPTPTPGCTSQKWAQCGGIGFSGCTTCVSGTTCQKLNDYYSQCL